European Patent Application EP 4 342 983 A1, published March 27, 2024. Title: METHOD FOR MODIFYING CELL. Applicant: CELLS & GENES BIOTECH (SHANGHAI) CO., LTD. The sequence listing filed with the application follows.

SEQUENCE LISTING (28 sequences)

SEQ ID NO: 1 - protein, 241 aa, Artificial Sequence
  Amino acid sequence of GFP protein
MVSKGEELFTGVVPILVELDGDVNGHKFSVSGEGEGDATYGKLTLKFICTTGKLPVPWPTLVTTLTYGVQCFSRYPDHMKQHDFFKSAMPEGYVQERTIFFKDDGNYKTRAEVKFEGDTLVNRIELKGIDFKEDGNILGHKLEYNYNSHNVYIMADKQKNGIKVNFKIRHNIEDGSVQLADHYQQNTPIGDGPVLLPDNHYLSTQSALSKDPNEKRDHMVLLEFVTAAGITLGMDELYKRS

SEQ ID NO: 2 - DNA, 799 bp, Artificial Sequence
  5' nucleic acid sequence homologous to human TRAC gene in plasmid 5
actctatcacggccatattctggcagggtcagtggctccaactaacatttgtttggtactttacagtttattaaatagatgtttatatggagaagctctcatttctttctcagaagagcctggctaggaaggtggatgaggcaccatattcattttgcaggtgaaattcctgagatgtaaggagctgctgtgacttgctcaaggccttatatcgagtaaacggtagtgctggggcttagacgcaggtgttctgatttatagttcaaaacctctatcaatgagagagcaatctcctggtaatgtgatagatttcccaacttaatgccaacataccataaacctcccattctgctaatgcccagcctaagttggggagaccactccagattccaagatgtacagtttgctttgctgggcctttttcccatgcctgcctttactctgccagagttatattgctggggttttgaagaagatcctattaaataaaagaataagcagtattattaagtagccctgcatttcaggtttccttgagtggcaggccaggcctggccgtgaacgttcactgaaatcatggcctcttggccaagattgatagcttgtgcctgtccctgagtcccagtccatcacgagcagctggtttctaagatgctatttcccgtataaagcatgagaccgtgacttgccagccccacagagccccgcccttgtccatcactggcatctggactccagcctgggttggggcaaagagggaaatgagatcatgtcctaaccctgatcctcttgtcccaca

SEQ ID NO: 3 - DNA, 801 bp, Artificial Sequence
  3' nucleic acid sequence homologous to human TRAC gene in plasmid 5
gatatccagaaccctgaccctgccgtgtaccagctgagagactctaaatccagtgacaagtctgtctgcctattcaccgattttgattctcaaacaaatgtgtcacaaagtaaggattctgatgtgtatatcacagacaaaactgtgctagacatgaggtctatggacttcaagagcaacagtgctgtggcctggagcaacaaatctgactttgcatgtgcaaacgccttcaacaacagcattattccagaagacaccttcttccccagcccaggtaagggcagctttggtgccttcgcaggctgtttccttgcttcaggaatggccaggttctgcccagagctctggtcaatgatgtctaaaactcctctgattggtggtctcggccttatccattgccaccaaaaccctctttttactaagaaacagtgagccttgttctggcagtccagagaatgacacgggaaaaaagcagatgaagagaaggtggcaggagagggcacgtggcccagcctcagtctctccaactgagttcctgcctgcctgcctttgctcagactgtttgccccttactgctcttctaggcctcattctaagccccttctccaagttgcctctccttatttctccctgtctgccaaaaaatctttcccagctcactaagtcagtctcacgcagtcactcattaacccaccaatcactgattgtgccggcacatgaatgcaccaggtgttgaagtggaggaattaaaaagtcagatgaggggtgtgcccagaggaagcaccattctagttgggggag

SEQ ID NO: 4 - DNA, 400 bp, Artificial Sequence
  5' nucleic acid sequence homologous to human TRAC gene in plasmid
cagtttgctttgctgggcctttttcccatgcctgcctttactctgccagagttatattgctggggttttgaagaagatcctattaaataaaagaataagcagtattattaagtagccctgcatttcaggtttccttgagtggcaggccaggcctggccgtgaacgttcactgaaatcatggcctcttggccaagattgatagcttgtgcctgtccctgagtcccagtccatcacgagcagctggtttctaagatgctatttcccgtataaagcatgagaccgtgacttgccagccccacagagccccgcccttgtccatcactggcatctggactccagcctgggttggggcaaagagggaaatgagatcatgtcctaaccctgatcctcttgtcccaca

SEQ ID NO: 5 - DNA, 400 bp, Artificial Sequence
  5' nucleic acid sequence homologous to human TRAC gene in plasmid
gatatccagaaccctgaccctgccgtgtaccagctgagagactctaaatccagtgacaagtctgtctgcctattcaccgattttgattctcaaacaaatgtgtcacaaagtaaggattctgatgtgtatatcacagacaaaactgtgctagacatgaggtctatggacttcaagagcaacagtgctgtggcctggagcaacaaatctgactttgcatgtgcaaacgccttcaacaacagcattattccagaagacaccttcttccccagcccaggtaagggcagctttggtgccttcgcaggctgtttccttgcttcaggaatggccaggttctgcccagagctctggtcaatgatgtctaaaactcctctgattggtggtctcggccttatccattgcc

SEQ ID NO: 6 - DNA, 300 bp, Artificial Sequence
  5' nucleic acid sequence homologous to human TRAC gene in plasmid 7
agtattattaagtagccctgcatttcaggtttccttgagtggcaggccaggcctggccgtgaacgttcactgaaatcatggcctcttggccaagattgatagcttgtgcctgtccctgagtcccagtccatcacgagcagctggtttctaagatgctatttcccgtataaagcatgagaccgtgacttgccagccccacagagccccgcccttgtccatcactggcatctggactccagcctgggttggggcaaagagggaaatgagatcatgtcctaaccctgatcctcttgtcccaca

SEQ ID NO: 7 - DNA, 300 bp, Artificial Sequence
  3' nucleic acid sequence homologous to human TRAC gene in plasmid 7
gatatccagaaccctgaccctgccgtgtaccagctgagagactctaaatccagtgacaagtctgtctgcctattcaccgattttgattctcaaacaaatgtgtcacaaagtaaggattctgatgtgtatatcacagacaaaactgtgctagacatgaggtctatggacttcaagagcaacagtgctgtggcctggagcaacaaatctgactttgcatgtgcaaacgccttcaacaacagcattattccagaagacaccttcttccccagcccaggtaagggcagctttggtgccttcgca

SEQ ID NO: 8 - DNA, 20 bp, Artificial Sequence
  sgRNA targeting human TRAC gene
tcagggttctggatatctgt

SEQ ID NO: 9 - protein, 489 aa, Artificial Sequence
  Amino acid sequence of CD19 CAR
MALPVTALLLPLALLLHAARPDIQMTQTTSSLSASLGDRVTISCRASQDISKYLNWYQQKPDGTVKLLIYHTSRLHSGVPSRFSGSGSGTDYSLTISNLEQEDIATYFCQQGNTLPYTFGGGTKLEITGSTSGSGKPGSGEGSTKGEVKLQESGPGLVAPSQSLSVTCTVSGVSLPDYGVSWIRQPPRKGLEWLGVIWGSETTYYNSALKSRLTIIKDNSKSQVFLKMNSLQTDDTAIYYCAKHYYYGGSYAMDYWGQGTSVTVSSTTTPAPRPPTPAPTIASQPLSLRPEACRPAAGGAVHTRGLDFACDIYIWAPLAGTCGVLLLSLVITLYCKRGRKKLLYIFKQPFMRPVQTTQEEDGCSCRFPEEEEGGCELRVKFSRSADAPAYQQGQNQLYNELNLGRREEYDVLDKRRGRDPEMGGKPRRKNPQEGLYNELQKDKMAEAYSEIGMKGERRRGKGHDGLYQGLSTATKDTYDALHMQALPPR

SEQ ID NO: 10 - protein, 245 aa, Artificial Sequence
  Amino acid sequence of scFv region targeting CD19
DIQMTQTTSSLSASLGDRVTISCRASQDISKYLNWYQQKPDGTVKLLIYHTSRLHSGVPSRFSGSGSGTDYSLTISNLEQEDIATYFCQQGNTLPYTFGGGTKLEITGSTSGSGKPGSGEGSTKGEVKLQESGPGLVAPSQSLSVTCTVSGVSLPDYGVSWIRQPPRKGLEWLGVIWGSETTYYNSALKSRLTIIKDNSKSQVFLKMNSLQTDDTAIYYCAKHYYYGGSYAMDYWGQGTSVTVSS

SEQ ID NO: 11 - protein, 486 aa, Artificial Sequence
  Amino acid sequence of GPC3 CAR
MALPVTALLLPLALLLHAARPQVQLVQSGAEVKKPGASVKVSCKASGYTFTDYEMHWVRQAPGQGLEWMGALDPKTGDTAYSQKFKGRVTLTADKSTSTAYMELSSLTSEDTAVYYCTRFYSYTYWGQGTLVTVSSGGGGSGGGGSGGGGSDVVMTQSPLSLPVTPGEPASISCRSSQSLVHSNGNTYLHWYLQKPGQSPQLLIYKVSNRFSGVPDRFSGSGSGTDFTLKISRVEAEDVGVYYCSQNTHVPPTFGQGTKLEIKTTTPAPRPPTPAPTIASQPLSLRPEACRPAAGGAVHTRGLDFACDIYIWAPLAGTCGVLLLSLVITLYCKRGRKKLLYIFKQPFMRPVQTTQEEDGCSCRFPEEEEGGCELRVKFSRSADAPAYQQGQNQLYNELNLGRREEYDVLDKRRGRDPEMGGKPRRKNPQEGLYNELQKDKMAEAYSEIGMKGERRRGKGHDGLYQGLSTATKDTYDALHMQALPPR

SEQ ID NO: 12 - protein, 242 aa, Artificial Sequence
  Amino acid sequence of scFv region targeting GPC3
QVQLVQSGAEVKKPGASVKVSCKASGYTFTDYEMHWVRQAPGQGLEWMGALDPKTGDTAYSQKFKGRVTLTADKSTSTAYMELSSLTSEDTAVYYCTRFYSYTYWGQGTLVTVSSGGGGSGGGGSGGGGSDVVMTQSPLSLPVTPGEPASISCRSSQSLVHSNGNTYLHWYLQKPGQSPQLLIYKVSNRFSGVPDRFSGSGSGTDFTLKISRVEAEDVGVYYCSQNTHVPPTFGQGTKLEIK

SEQ ID NO: 13 - protein, 645 aa, Artificial Sequence
  Amino acid sequence of CD19 CAR-2A-IL15
MALPVTALLLPLALLLHAARPDIQMTQTTSSLSASLGDRVTISCRASQDISKYLNWYQQKPDGTVKLLIYHTSRLHSGVPSRFSGSGSGTDYSLTISNLEQEDIATYFCQQGNTLPYTFGGGTKLEITGSTSGSGKPGSGEGSTKGEVKLQESGPGLVAPSQSLSVTCTVSGVSLPDYGVSWIRQPPRKGLEWLGVIWGSETTYYNSALKSRLTIIKDNSKSQVFLKMNSLQTDDTAIYYCAKHYYYGGSYAMDYWGQGTSVTVSSTTTPAPRPPTPAPTIASQPLSLRPEACRPAAGGAVHTRGLDFACDIYIWAPLAGTCGVLLLSLVITLYCKRGRKKLLYIFKQPFMRPVQTTQEEDGCSCRFPEEEEGGCELRVKFSRSADAPAYQQGQNQLYNELNLGRREEYDVLDKRRGRDPEMGGKPRRKNPQEGLYNELQKDKMAEAYSEIGMKGERRRGKGHDGLYQGLSTATKDTYDALHMQALPPRGSGATNFSLLKQAGDVEENPGPMGWSCIILFLVATATGVHSMNWVNVISDLKKIEDLIQSMHIDATLYTESDVHPSCKVTAMKCFLLELQVISLESGDASIHDTVENLIILANNSLSSNGNVTESGCKECEELEEKNIKEFLQSFVHIVQMFINTS

SEQ ID NO: 14 - protein, 498 aa, Artificial Sequence
  Amino acid sequence of BiTE
DIQLTQSPASLAVSLGQRATISCKASQSVDYDGDSYLNWYQQIPGQPPKLLIYDASNLVSGIPPRFSGSGSGTDFTLNIHPVEKVDAATYHCQQSTEDPWTFGGGTKLEIKGGGGSGGGGSGGGGSQVQLQQSGAELVRPGSSVKISCKASGYAFSSYWMNWVKQRPGQGLEWIGQIWPGDGDTNYNGKFKGKATLTADESSSTAYMQLSSLASEDSAVYFCARRETTTVGRYYYAMDYWGQGTTVTVSSGGGGSDIKLQQSGAELARPGASVKMSCKTSGYTFTRYTMHWVKQRPGQGLEWIGYINPSRGYTNYNQKFKDKATLTTDKSSSTAYMQLSSLTSEDSAVYYCARYYDDHYCLDYWGQGTTLTVSSVEGGSGGSGGSGGSGGVDDIQLTQSPAIMSASPGEKVTMTCRASSSVSYMNWYQQKSGTSPKRWIYDTSKVASGVPYRFSGSGSGTSYSLTISSMEAEDAATYYCQQWSSNPLTFGAGTKLELK

SEQ ID NO: 15 - protein, 1036 aa, Artificial Sequence
  Amino acid sequence of CD19 CAR-2A-BiTE
MALPVTALLLPLALLLHAARPDIQMTQTTSSLSASLGDRVTISCRASQDISKYLNWYQQKPDGTVKLLIYHTSRLHSGVPSRFSGSGSGTDYSLTISNLEQEDIATYFCQQGNTLPYTFGGGTKLEITGSTSGSGKPGSGEGSTKGEVKLQESGPGLVAPSQSLSVTCTVSGVSLPDYGVSWIRQPPRKGLEWLGVIWGSETTYYNSALKSRLTIIKDNSKSQVFLKMNSLQTDDTAIYYCAKHYYYGGSYAMDYWGQGTSVTVSSTTTPAPRPPTPAPTIASQPLSLRPEACRPAAGGAVHTRGLDFACDIYIWAPLAGTCGVLLLSLVITLYCKRGRKKLLYIFKQPFMRPVQTTQEEDGCSCRFPEEEEGGCELRVKFSRSADAPAYQQGQNQLYNELNLGRREEYDVLDKRRGRDPEMGGKPRRKNPQEGLYNELQKDKMAEAYSEIGMKGERRRGKGHDGLYQGLSTATKDTYDALHMQALPPRGSGATNFSLLKQAGDVEENPGPMGWSCIILFLVATATGVHSDYKDDDDKDIQLTQSPASLAVSLGQRATISCKASQSVDYDGDSYLNWYQQIPGQPPKLLIYDASNLVSGIPPRFSGSGSGTDFTLNIHPVEKVDAATYHCQQSTEDPWTFGGGTKLEIKGGGGSGGGGSGGGGSQVQLQQSGAELVRPGSSVKISCKASGYAFSSYWMNWVKQRPGQGLEWIGQIWPGDGDTNYNGKFKGKATLTADESSSTAYMQLSSLASEDSAVYFCARRETTTVGRYYYAMDYWGQGTTVTVSSGGGGSDIKLQQSGAELARPGASVKMSCKTSGYTFTRYTMHWVKQRPGQGLEWIGYINPSRGYTNYNQKFKDKATLTTDKSSSTAYMQLSSLTSEDSAVYYCARYYDDHYCLDYWGQGTTLTVSSVEGGSGGSGGSGGSGGVDDIQLTQSPAIMSASPGEKVTMTCRASSSVSYMNWYQQKSGTSPKRWIYDTSKVASGVPYRFSGSGSGTSYSLTISSMEAEDAATYYCQQWSSNPLTFGAGTKLELK

SEQ ID NO: 16 - protein, 670 aa, Artificial Sequence
  Amino acid sequence of GPC3 CAR-2A-IL15
MALPVTALLLPLALLLHAARPQVQLVQSGAEVKKPGASVKVSCKASGYTFTDYEMHWVRQAPGQGLEWMGALDPKTGDTAYSQKFKGRVTLTADKSTSTAYMELSSLTSEDTAVYYCTRFYSYTYWGQGTLVTVSSGGGGSGGGGSGGGGSDVVMTQSPLSLPVTPGEPASISCRSSQSLVHSNGNTYLHWYLQKPGQSPQLLIYKVSNRFSGVPDRFSGSGSGTDFTLKISRVEAEDVGVYYCSQNTHVPPTFGQGTKLEIKTTTPAPRPPTPAPTIASQPLSLRPEACRPAAGGAVHTRGLDFACDIYIWAPLAGTCGVLLLSLVITLYCKRGRKKLLYIFKQPFMRPVQTTQEEDGCSCRFPEEEEGGCELRVKFSRSADAPAYQQGQNQLYNELNLGRREEYDVLDKRRGRDPEMGGKPRRKNPQEGLYNELQKDKMAEAYSEIGMKGERRRGKGHDGLYQGLSTATKDTYDALHMQALPPRGSGATNFSLLKQAGDVEENPGPMRISKPHLRSISIQCYLCLLLNSHFLTEAGIHVFILGCFSAGLPKTEANWVNVISDLKKIEDLIQSMHIDATLYTESDVHPSCKVTAMKCFLLELQVISLESGDASIHDTVENLIILANNSLSSNGNVTESGCKECEELEEKNIKEFLQSFVHIVQMFINTS

SEQ ID NO: 17 - protein, 808 aa, Artificial Sequence
  Amino acid sequence of GPC3 CAR-2A-IL7-2A-CCL19
MALPVTALLLPLALLLHAARPQVQLVQSGAEVKKPGASVKVSCKASGYTFTDYEMHWVRQAPGQGLEWMGALDPKTGDTAYSQKFKGRVTLTADKSTSTAYMELSSLTSEDTAVYYCTRFYSYTYWGQGTLVTVSSGGGGSGGGGSGGGGSDVVMTQSPLSLPVTPGEPASISCRSSQSLVHSNGNTYLHWYLQKPGQSPQLLIYKVSNRFSGVPDRFSGSGSGTDFTLKISRVEAEDVGVYYCSQNTHVPPTFGQGTKLEIKTTTPAPRPPTPAPTIASQPLSLRPEACRPAAGGAVHTRGLDFACDIYIWAPLAGTCGVLLLSLVITLYCKRGRKKLLYIFKQPFMRPVQTTQEEDGCSCRFPEEEEGGCELRVKFSRSADAPAYQQGQNQLYNELNLGRREEYDVLDKRRGRDPEMGGKPRRKNPQEGLYNELQKDKMAEAYSEIGMKGERRRGKGHDGLYQGLSTATKDTYDALHMQALPPRGSGATNFSLLKQAGDVEENPGPMFHVSFRYIFGLPPLILVLLPVASSDCDIEGKDGKQYESVLMVSIDQLLDSMKEIGSNCLNNEFNFFKRHICDANKEGMFLFRAARKLRQFLKMNSTGDFDLHLLKVSEGTTILLNCTGQVKGRKPAALGEAQPTKSLEENKSLKEQKKLNDLCFLKRLLQEIKTCWNKILMGTKEHGSGVKQTLNFDLLKLAGDVESNPGPMALLLALSLLVLWTSPAPTLSGTNDAEDCCLSVTQKPIPGYIVRNFHYLLIKDGCRVPAVVFTTLRGRQLCAPPDQPWVERIIQRLQRTSAKMKRRSS

SEQ ID NO: 18 - DNA, 20 bp, Artificial Sequence
  sgRNA targeting AAVS-1
ggggccactagggacaggat

SEQ ID NO: 19 - DNA, 309 bp, Artificial Sequence
  DNA sequence
ctcctgtggattcgggtcacctctcactcctttcatttgggcagctcccctaccccccttacctctctagtctgtgctagctcttccagccccctgtcatggcatcttccaggggtccgagagctcagctagtcttcttcctccaacccgggcccctatgtccacttcaggacagcatgtttgctgcctccagggatcctgtgtccccgagctgggaccaccttatattcccagggccggttaatgtggctctggttctgggtacttttatctgtcccctccaccccacagtggggccactagggacag

SEQ ID NO: 20 - DNA, 327 bp, Artificial Sequence
  DNA sequence
gattggtgacagaaaagccccatccttaggcctcctccttcctagtctcctgatattgggtctaacccccacctcctgttaggcagattccttatctggtgacacacccccatttcctggagccatctctctccttgccagaacctctaaggtttgcttacgatggagccagagaggatcctgggagggagagcttggcagggggtgggagggaagggggggatgcgtgacctgcccggttctcagtggccaccctgcgctaccctctcccagaacctgagctgctctgacgcggctgtctggtgcgtttcactgatcctggtgctg

SEQ ID NO: 21 - DNA, 23 bp, Artificial Sequence
  Forward primer
tgagtcccagtccatcacgagca

SEQ ID NO: 22 - DNA, 22 bp, Artificial Sequence
  Reverse primer
ggactgccagaacaaggctcac

SEQ ID NO: 23 - DNA, 21 bp, Artificial Sequence
  Forward primer
agcactgcctctgtcactctc

SEQ ID NO: 24 - DNA, 21 bp, Artificial Sequence
  Reverse primer
acttgggccaggggaggagtt

SEQ ID NO: 25 - DNA, 20 bp, Artificial Sequence
  sgRNA targeting PD-1
ggccaggatggttcttaggt

SEQ ID NO: 26 - DNA, 20 bp, Artificial Sequence
  Forward primer
cgttccccagcgaggcttcc

SEQ ID NO: 27 - DNA, 21 bp, Artificial Sequence
  Reverse primer
cgggcctgagggaaggtccta

SEQ ID NO: 28 - DNA, 20 bp, Artificial Sequence
  sgRNA targeting CD95
gagggtccagatgcccagca